European Patent Specification EP 4 222 500 B1, published November 12, 2025. Title: METHODS OF DETECTING ISOASPARTIC ACID. Applicant: Amgen Inc. The sequence listing filed with the application follows.

SEQUENCE LISTING (27 sequences)

SEQ ID NO: 1 - protein, 9 aa, Artificial Sequence
  Synthetic Polypeptide
  MISC_FEATURE (5)..(5): ISO
WAGGDASGE

SEQ ID NO: 2 - protein, 9 aa, Artificial Sequence
  Synthetic Polypeptide
WAGGDASGE

SEQ ID NO: 3 - protein, 26 aa, Artificial Sequence
  Synthetic Polypeptide
WGGDGFYAMDYWGQGTLVTVSSASTK

SEQ ID NO: 4 - protein, 10 aa, Artificial Sequence
  Synthetic Polypeptide
CSRWGGDGFY

SEQ ID NO: 5 - protein, 6 aa, Artificial Sequence
  Synthetic Polypeptide
  MISC_FEATURE (3)..(3): ISO
VTDNVK

SEQ ID NO: 6 - protein, 26 aa, Artificial Sequence
  Synthetic Polypeptide
  MISC_FEATURE (4)..(4): ISO
WGGDGFYAMDYWGQGTLVTVSSASTK

SEQ ID NO: 7 - protein, 10 aa, Artificial Sequence
  Synthetic Polypeptide
  MISC_FEATURE (7)..(7): ISO
CSRWGGDGFY

SEQ ID NO: 8 - protein, 5 aa, Artificial Sequence
  Synthetic Polypeptide
ALDGE

SEQ ID NO: 9 - protein, 5 aa, Artificial Sequence
  Synthetic Polypeptide
  MISC_FEATURE (3)..(3): ISO
ALDGE

SEQ ID NO: 10 - protein, 5 aa, Artificial Sequence
  Synthetic Polypeptide
ALDEK

SEQ ID NO: 11 - protein, 5 aa, Artificial Sequence
  Synthetic Polypeptide
  MISC_FEATURE (3)..(3): ISO
ALDEK

SEQ ID NO: 12 - protein, 5 aa, Artificial Sequence
  Synthetic Polypeptide
ALDGK

SEQ ID NO: 13 - protein, 5 aa, Artificial Sequence
  Synthetic Polypeptide
  MISC_FEATURE (3)..(3): ISO
ALDGK

SEQ ID NO: 14 - protein, 6 aa, Artificial Sequence
  Synthetic Polypeptide
GLDLLK

SEQ ID NO: 15 - protein, 6 aa, Artificial Sequence
  Synthetic Polypeptide
  MISC_FEATURE (3)..(3): ISO
GLDLLK

SEQ ID NO: 16 - protein, 6 aa, Artificial Sequence
  Synthetic Polypeptide
GDLLLK

SEQ ID NO: 17 - protein, 6 aa, Artificial Sequence
  Synthetic Polypeptide
  MISC_FEATURE (2)..(2): ISO
GDLLLK

SEQ ID NO: 18 - protein, 15 aa, Artificial Sequence
  Synthetic Polypeptide
VVSLTVLHQDWLNGK

SEQ ID NO: 19 - protein, 15 aa, Artificial Sequence
  Synthetic Polypeptide
  MISC_FEATURE (10)..(10): ISO
VVSLTVLHQDWLNGK

SEQ ID NO: 20 - protein, 22 aa, Artificial Sequence
  Synthetic Polypeptide
GFYPSDIAVEWESDGQPENNYK

SEQ ID NO: 21 - protein, 22 aa, Artificial Sequence
  Synthetic Polypeptide
  MISC_FEATURE (14)..(14): ISO
GFYPSDIAVEWESDGQPENNYK

SEQ ID NO: 22 - protein, 5 aa, Artificial Sequence
  Synthetic Polypeptide
ADLGK

SEQ ID NO: 23 - protein, 5 aa, Artificial Sequence
  Synthetic Polypeptide
  MISC_FEATURE (2)..(2): ISO
ADLGK

SEQ ID NO: 24 - protein, 22 aa, Artificial Sequence
  Synthetic Polypeptide
GFYPSDIAVEWESNGQPEDNYK

SEQ ID NO: 25 - protein, 22 aa, Artificial Sequence
  Synthetic Polypeptide
  MISC_FEATURE (19)..(19): ISO
GFYPSDIAVEWESNGQPEDNYK

SEQ ID NO: 26 - protein, 22 aa, Artificial Sequence
  Synthetic Polypeptide
GFYPSDIAVEWESNGQPENDYK

SEQ ID NO: 27 - protein, 22 aa, Artificial Sequence
  Synthetic Polypeptide
  MISC_FEATURE (20)..(20): ISO
GFYPSDIAVEWESNGQPENDYK